European Patent Application EP 4 789 715 A2, published August 12, 2026. Title: METHODS FOR TREATING NEOINTIMAL HYPERPLASIA USING F11R/JAM-A INHIBITORS. Applicant: The Research Foundation for The State University of New York. The sequence listing filed with the application follows.

SEQUENCE LISTING (17 sequences)

SEQ ID NO: 1 - protein, 13 aa, synthetic construct
  REGION 1..13: note = Laboratory synthesized sequence
  SITE 1: note = MISC_FEATURE - Xaa is Lysine or D-Lysine
  SITE 5: note = MISC_FEATURE - Xaa is Arginine or D-Arginine
  MOD_RES 13: note = optionally amidated cysteine
XSVTXEDTGTYTC

SEQ ID NO: 2 - protein, 13 aa, synthetic construct
  REGION 1..13: note = Laboratory synthesized sequence
KSVTREDTGTYTC

SEQ ID NO: 3 - protein, 13 aa, synthetic construct
  REGION 1..13: note = Laboratory synthesized sequence
  SITE 1: note = MISC_FEATURE - Xaa is D-Lysine
  SITE 5: note = MISC_FEATURE - Xaa is D-Arginine
  MOD_RES 13: note = amidated cysteine
XSVTXEDTGTYTC

SEQ ID NO: 4 - protein, 13 aa, synthetic construct
  REGION 1..13: note = Laboratory synthesized sequence
  MOD_RES 13: note = amidated cysteine
KSVTREDTGTYTC

SEQ ID NO: 5 - protein, 13 aa, synthetic construct
  REGION 1..13: note = Laboratory synthesized sequence
  SITE 5: note = MISC_FEATURE - Xaa is D-Arginine
  MOD_RES 13: note = amidated cysteine
KSVTXEDTGTYTC

SEQ ID NO: 6 - protein, 13 aa, synthetic construct
  REGION 1..13: note = Laboratory synthesized sequence
  SITE 1: note = MISC_FEATURE - Xaa is D-Lysine
  MOD_RES 13: note = amidated cysteine
XSVTREDTGTYTC

SEQ ID NO: 7 - protein, 13 aa, synthetic construct
  REGION 1..13: note = Laboratory synthesized sequence
  SITE 5: note = MISC_FEATURE - Xaa is D-Arginine
KSVTXEDTGTYTC

SEQ ID NO: 8 - protein, 13 aa, synthetic construct
  REGION 1..13: note = Laboratory synthesized sequence
  SITE 1: note = MISC_FEATURE - Xaa is D-Lysine
XSVTREDTGTYTC

SEQ ID NO: 9 - protein, 13 aa, synthetic construct
  REGION 1..13: note = Laboratory synthesized sequence
  SITE 1: note = MISC_FEATURE - Xaa is D-Lysine
  SITE 5: note = MISC_FEATURE - Xaa is D-Arginine
XSVTXEDTGTYTC

SEQ ID NO: 10 - protein, 23 aa, synthetic construct
  REGION 1..23: note = Laboratory synthesized sequence
  SITE 12: note = MISC_FEATURE - Xaa is Arginine or D-Arginine
  MOD_RES 23: note = optionally amidated cysteine
SVTVHSSEPEVXIPENNPVKLSC

SEQ ID NO: 11 - protein, 23 aa, synthetic construct
  REGION 1..23: note = Laboratory synthesized sequence
  SITE 12: note = misc_feature - Xaa can be any naturally occurring amino acid
SVTVHSSEPEVXIPENNPVKLSC

SEQ ID NO: 12 - protein, 23 aa, synthetic construct
  REGION 1..23: note = Laboratory synthesized sequence
  MOD_RES 23: note = amidated cysteine
SVTVHSSEPEVRIPENNPVKLSC

SEQ ID NO: 13 - protein, 23 aa, synthetic construct
  REGION 1..23: note = Laboratory synthesized sequence
  SITE 12: note = MISC_FEATURE - Xaa is D-Arginine
SVTVHSSEPEVXIPENNPVKLSC

SEQ ID NO: 14 - protein, 23 aa, synthetic construct
  REGION 1..23: note = Laboratory synthesized sequence
  SITE 12: note = MISC_FEATURE - Xaa is D-Arginine
  MOD_RES 23: note = amidated cysteine
SVTVHSSEPEVXIPENNPVKLSC

SEQ ID NO: 15 - protein, 14 aa, synthetic construct
  REGION 1..14: note = Laboratory synthesized sequence
  SITE 7: note = MISC_FEATURE - Xaa is Arginine or D-Arginine
SSEPEVXIPENNPV

SEQ ID NO: 16 - protein, 14 aa, synthetic construct
  REGION 1..14: note = Laboratory synthesized sequence
SSEPEVRIPENNPV

SEQ ID NO: 17 - protein, 14 aa, synthetic construct
  REGION 1..14: note = Laboratory synthesized sequence
  SITE 7: note = MISC_FEATURE - Xaa is D-Arginine
SSEPEVXIPENNPV